European Patent Specification EP 3 674 328 B1, published December 13, 2023. Title: CHIMERIC ANTIGEN RECEPTOR (CAR) BINDING TO BCMA, AND USES THEREOF. Applicant: NANJING IASO BIOTHERAPEUTICS CO., LTD.; INNOVENT BIOLOGICS (SUZHOU) CO., LTD. The sequence listing filed with the application follows.

SEQUENCE LISTING (52 sequences)

SEQ ID NO: 1 - protein, 3 aa, Artificial Sequence
  KOZAK
AAT

SEQ ID NO: 2 - DNA, 9 bp, Artificial Sequence
  KOZAK (nucleotide)
gccgccacc

SEQ ID NO: 3 - protein, 21 aa, Artificial Sequence
  CD8a signal peptide
MALPVTALLLPLALLLHAARP

SEQ ID NO: 4 - DNA, 63 bp, Artificial Sequence
  CD8a signal peptide (nucleotide)
atggccctgcctgtgacagctctgctcctccctctggccctgctgctccatgccgccagaccc

SEQ ID NO: 5 - protein, 9 aa, Artificial Sequence
  HA-tag
YPYDVPDYA

SEQ ID NO: 6 - DNA, 27 bp, Artificial Sequence
  HA-tag (nucleotide)
tacccatacgatgttccagattacgct

SEQ ID NO: 7 - protein, 119 aa, Artificial Sequence
  VH
QLQLQESGPGLVKPSETLSLTCTVSGGSISSSSYYWGWIRQPPGKGLEWIGSISYSGSTYYNPSLKSRVTISVDTSKNQFSLKLSSVTAADTAVYYCARDRGDTILDVWGQGTMVTVSS

SEQ ID NO: 8 - DNA, 357 bp, Artificial Sequence
  VH (nucleotide)
cagctgcagctgcaggagtcgggcccaggactggtgaagccttcggagaccctgtccctcacctgcactgtctctggtggctccatcagcagtagtagttactactggggctggatccgccagcccccagggaaggggctggagtggattgggagtatctcctatagtgggagcacctactacaacccgtccctcaagagtcgagtcaccatatccgtagacacgtccaagaaccagttctccctgaagctgagttctgtgaccgccgcagacacggcggtgtactactgcgccagagatcgtggagacaccatactagacgtatggggtcagggtacaatggtcaccgtcagctca

SEQ ID NO: 9 - protein, 10 aa, Artificial Sequence
  HCDR1
GGSISSSSYY

SEQ ID NO: 10 - protein, 7 aa, Artificial Sequence
  HCDR2
ISYSGST

SEQ ID NO: 11 - protein, 11 aa, Artificial Sequence
  HCDR3
ARDRGDTILDV

SEQ ID NO: 12 - DNA, 30 bp, Artificial Sequence
  HCDR1 (nucleotide)
ggtggctccatcagcagtagtagttactac

SEQ ID NO: 13 - DNA, 21 bp, Artificial Sequence
  HCDR2 (nucleotide)
atctcctatagtgggagcacc

SEQ ID NO: 14 - DNA, 33 bp, Artificial Sequence
  HCDR3 (nucleotide)
gccagagatcgtggagacaccatactagacgta

SEQ ID NO: 15 - protein, 106 aa, Artificial Sequence
  VL
DIQMTQSPSSLSASVGDRVTITCRASQSISSYLNWYQQKPGKAPKLLIYAASSLQSGVPSRFSGSGSGTDFTLTISSLQPEDFATYYCQQKYDLLTFGGGTKVEIK

SEQ ID NO: 16 - DNA, 318 bp, Artificial Sequence
  VL (nucleotide)
gacatccagatgacccagtctccatcctccctgtctgcatctgtaggagacagagtcaccatcacttgccgggcaagtcagagcattagcagctatttaaattggtatcagcagaaaccagggaaagcccctaagctcctgatctatgctgcatccagtttgcaaagtggggtcccatcaaggttcagtggcagtggatctgggacagatttcactctcaccatcagcagtctgcaacctgaagattttgcaacttactactgtcagcaaaaatacgacctcctcacttttggcggagggaccaaggttgagatcaaa

SEQ ID NO: 17 - protein, 6 aa, Artificial Sequence
  LCDR1
QSISSY

SEQ ID NO: 18 - protein, 3 aa, Artificial Sequence
  LCDR2
AAS

SEQ ID NO: 19 - protein, 8 aa, Artificial Sequence
  LCDR3
QQKYDLLT

SEQ ID NO: 20 - DNA, 18 bp, Artificial Sequence
  LCDR1 (nucleotide)
cagagcattagcagctat

SEQ ID NO: 21 - DNA, 9 bp, Artificial Sequence
  LCDR2 (nucleotide)
gctgcatcc

SEQ ID NO: 22 - DNA, 24 bp, Artificial Sequence
  LCDR3 (nucleotide)
cagcaaaaatacgacctcctcact

SEQ ID NO: 23 - protein, 18 aa, Artificial Sequence
  Linker (VL-VH)
GSTSGSGKPGSGEGSTKG

SEQ ID NO: 24 - DNA, 54 bp, Artificial Sequence
  Linker (VL-VH) (nucleotide)
ggcagcaccagcggctccggcaagcctggctctggcgagggcagcacaaaggga

SEQ ID NO: 25 - protein, 55 aa, Artificial Sequence
  Structural domain
FVPVFLPAKPTTTPAPRPPTPAPTIASQPLSLRPEACRPAAGGAVHTRGLDFACD

SEQ ID NO: 26 - DNA, 165 bp, Artificial Sequence
  Structural domain (nucleotide)
ttcgtgcccgtgttcctgcccgccaaacctaccaccacccctgcccctagacctcccaccccagccccaacaatcgccagccagcctctgtctctgcggcccgaagcctgtagacctgctgccggcggagccgtgcacaccagaggcctggacttcgcctgcgac

SEQ ID NO: 27 - protein, 21 aa, Artificial Sequence
  CD8a transmembrane domain
IYIWAPLAGTCGVLLLSLVIT

SEQ ID NO: 28 - DNA, 63 bp, Artificial Sequence
  CD8a transmembrane domain (nucleotide)
atctacatctgggcccctctggccggcacctgtggcgtgctgctgctgagcctggtgatcacc

SEQ ID NO: 29 - protein, 41 aa, Artificial Sequence
  CD28 costimulatory domain
RSKRSRLLHSDYMNMTPRRPGPTRKHYQPYAPPRDFAAYRS

SEQ ID NO: 30 - DNA, 123 bp, Artificial Sequence
  CD28 costimulatory domain (nucleotide)
agaagcaagcggagccggctgctgcacagcgactacatgaacatgaccccaagacggcctggccccacccggaagcactaccagccttacgcccctcccagagacttcgccgcctaccggtcc

SEQ ID NO: 31 - protein, 42 aa, Artificial Sequence
  4-1BB costimulatory domain
KRGRKKLLYIFKQPFMRPVQTTQEEDGCSCRFPEEEEGGCEL

SEQ ID NO: 32 - DNA, 126 bp, Artificial Sequence
  4-1BB costimulatory domain (nucleotide)
aaacggggcagaaagaaactcctgtatatattcaaacaaccatttatgagaccagtacaaactactcaagaggaagatggctgtagctgccgatttccagaagaagaagaaggaggatgtgaactg

SEQ ID NO: 33 - protein, 112 aa, Artificial Sequence
  CD3zeta intracellular signal transduction domain
RVKFSRSADAPAYQQGQNQLYNELNLGRREEYDVLDKRRGRDPEMGGKPRRKNPQEGLYNELQKDKMAEAYSEIGMKGERRRGKGHDGLYQGLSTATKDTYDALHMQALPPR

SEQ ID NO: 34 - DNA, 336 bp, Artificial Sequence
  CD3zeta intracellular signal transduction domain (nucleotide)
agagtgaagttcagcagatccgccgacgcccctgcctaccagcagggacagaaccagctgtacaacgagctgaacctgggcagacgggaagagtacgacgtgctggacaagcggagaggccgggaccccgagatgggcggaaagcccagacggaagaacccccaggaaggcctgtataacgaactgcagaaagacaagatggccgaggcctacagcgagatcggcatgaagggcgagcggaggcgcggcaagggccacgatggcctgtaccagggcctgagcaccgccaccaaggacacctacgacgccctgcacatgcaggccctgccccccaga

SEQ ID NO: 35 - protein, 18 aa, Artificial Sequence
  cleaving peptide T2A
EGRGSLLTCGDVEENPGP

SEQ ID NO: 36 - DNA, 54 bp, Artificial Sequence
  cleaving peptide T2A (nucleotide)
gagggcagaggaagtcttctaacatgcggtgacgtggaggagaatcccggccct

SEQ ID NO: 37 - protein, 239 aa, Artificial Sequence
  GFP
MVSKGEELFTGVVPILVELDGDVNGHKFSVSGEGEGDATYGKLTLKFICTTGKLPVPWPTLVTTLTYGVQCFSRYPDHMKQHDFFKSAMPEGYVQERTIFFKDDGNYKTRAEVKFEGDTLVNRIELKGIDFKEDGNILGHKLEYNYNSHNVYIMADKQKNGIKVNFKIRHNIEDGSVQLADHYQQNTPIGDGPVLLPDNHYLSTQSALSKDPNEKRDHMVLLEFVTAAGITLGMDELYK

SEQ ID NO: 38 - DNA, 720 bp, Artificial Sequence
  GFP (nucleotide)
atggtgagcaagggcgaggagctgttcaccggggtggtgcccatcctggtcgagctggacggcgacgtaaacggccacaagttcagcgtgtccggcgagggcgagggcgatgccacctacggcaagctgaccctgaagttcatctgcaccaccggcaagctgcccgtgccctggcccaccctcgtgaccaccctgacctacggcgtgcagtgcttcagccgctaccccgaccacatgaagcagcacgacttcttcaagtccgccatgcccgaaggctacgtccaggagcgcaccatcttcttcaaggacgacggcaactacaagacccgcgccgaggtgaagttcgagggcgacaccctggtgaaccgcatcgagctgaagggcatcgacttcaaggaggacggcaacatcctggggcacaagctggagtacaactacaacagccacaacgtctatatcatggccgacaagcagaagaacggcatcaaggtgaacttcaagatccgccacaacatcgaggacggcagcgtgcagctcgccgaccactaccagcagaacacccccatcggcgacggccccgtgctgctgcccgacaaccactacctgagcacccagtccgccctgagcaaagaccccaacgagaagcgcgatcacatggtcctgctggagttcgtgaccgccgccgggatcactctcggcatggacgagctgtacaagtaa

SEQ ID NO: 39 - protein, 357 aa, Artificial Sequence
  EGFRt
MLLLVTSLLLCELPHPAFLLIPRKVCNGIGIGEFKDSLSINATNIKHFKNCTSISGDLHILPVAFRGDSFTHTPPLDPQELDILKTVKEITGFLLIQAWPENRTDLHAFENLEIIRGRTKQHGQFSLAVVSLNITSLGLRSLKEISDGDVIISGNKNLCYANTINWKKLFGTSGQKTKIISNRGENSCKATGQVCHALCSPEGCWGPEPRDCVSCRNVSRGRECVDKCNLLEGEPREFVENSECIQCHPECLPQAMNITCTGRGPDNCIQCAHYIDGPHCVKTCPAGVMGENNTLVWKYADAGHVCHLCHPNCTYGCTGPGLEGCPTNGPKIPSIATGMVGALLLLLVVALGIGLFM

SEQ ID NO: 40 - DNA, 1071 bp, Artificial Sequence
  EGFRt (nucleotide)
atgctgctgctcgtgacctctttactgttatgtgagctgccccaccccgcttttttactgatccctcgtaaggtgtgtaacggaatcggcattggcgagttcaaggactctttaagcatcaacgccacaaacatcaagcacttcaagaattgtacctccatcagcggcgatttacacattctccccgtggcttttcgtggcgattccttcacccacaccccccctctggacccccaagagctggacattttaaaaaccgtgaaggagatcaccggctttctgctgatccaagcttggcccgagaatcgtaccgacctccacgccttcgagaatttagagattattcgtggaaggaccaagcagcacggccagttctctttagccgtcgtgtctttaaacattaccagcctcggtttaaggtctttaaaggagattagcgacggcgacgtgatcatctccggcaacaagaacctctgctacgccaacaccatcaactggaagaagctgttcggaaccagcggccaaaagaccaagatcatcagcaatcgtggagagaactcttgtaaggccactggtcaagtttgccacgccctctgtagccccgaaggatgttggggccccgagcctagggactgtgttagctgcagaaacgtgagcagaggcagagagtgtgtggacaaatgcaatttactggaaggagagcctagggagttcgtggagaacagcgaatgtatccagtgccaccccgagtgtttacctcaagccatgaacatcacttgtaccggaaggggccccgataactgcatccaatgcgcccactacatcgacggaccccactgcgtgaaaacttgtcccgccggagtgatgggagagaataacactttagtgtggaagtacgccgacgctggccacgtctgccatctgtgccaccccaactgtacctacggctgcactggtcccggtttagagggatgtcctaccaacggccccaagatcccctccatcgccaccggaatggtgggcgctctgttattactgctggtggtggctctgggcatcggtttattcatg

SEQ ID NO: 41 - protein, 246 aa, Artificial Sequence
  scFv0008
DIVLTQSPPSLAMSLGKRATISCRASESVTILGSHLIHWYQQKPGQPPTLLIQLASNVQTGVPARFSGSGSRTDFTLTIDPVEEDDVAVYYCLQSRTIPRTFGGGTKLEIKGSTSGSGKPGSGEGSTKGQIQLVQSGPELKKPGETVKISCKASGYTFTDYSINWVKRAPGKGLKWMGWINTETREPAYAYDFRGRFAFSLETSASTAYLQINNLKYEDTATYFCALDYSYAMDYWGQGTSVTVSS

SEQ ID NO: 42 - DNA, 738 bp, Artificial Sequence
  scFv0008 (nucleotide)
gacatcgtgctgacccagagcccccccagcctggccatgtctctgggcaagagagccaccatcagctgccgggccagcgagagcgtgaccatcctgggcagccacctgatccactggtatcagcagaagcccggccagccccccaccctgctgatccagctcgccagcaatgtgcagaccggcgtgcccgccagattcagcggcagcggcagcagaaccgacttcaccctgaccatcgaccccgtggaagaggacgacgtggccgtgtactactgcctgcagagccggaccatcccccggacctttggcggaggcaccaaactggaaatcaagggcagcaccagcggctccggcaagcctggctctggcgagggcagcacaaagggacagattcagctggtgcagagcggccctgagctgaagaaacccggcgagacagtgaagatcagctgcaaggcctccggctacaccttcaccgactacagcatcaactgggtgaaaagagcccctggcaagggcctgaagtggatgggctggatcaacaccgagacaagagagcccgcctacgcctacgacttccggggcagattcgccttcagcctggaaaccagcgccagcaccgcctacctgcagatcaacaacctgaagtacgaggacaccgccacctacttttgcgccctggactacagctacgccatggactactggggccagggcaccagcgtgaccgtgtccagc

SEQ ID NO: 43 - protein, 243 aa, Artificial Sequence
  scFv0026
DIQMTQSPSSLSASVGDRVTITCRASQSISSYLNWYQQKPGKAPKLLIYAASSLQSGVPSRFSGSGSGTDFTLTISSLQPEDFATYYCQQKYDLLTFGGGTKVEIKGSTSGSGKPGSGEGSTKGQLQLQESGPGLVKPSETLSLTCTVSGGSISSSSYYWGWIRQPPGKGLEWIGSISYSGSTYYNPSLKSRVTISVDTSKNQFSLKLSSVTAADTAVYYCARDRGDTILDVWGQGTMVTVSS

SEQ ID NO: 44 - DNA, 729 bp, Artificial Sequence
  scFv0026 (nucleotide)
gacatccagatgacccagtctccatcctccctgtctgcatctgtaggagacagagtcaccatcacttgccgggcaagtcagagcattagcagctatttaaattggtatcagcagaaaccagggaaagcccctaagctcctgatctatgctgcatccagtttgcaaagtggggtcccatcaaggttcagtggcagtggatctgggacagatttcactctcaccatcagcagtctgcaacctgaagattttgcaacttactactgtcagcaaaaatacgacctcctcacttttggcggagggaccaaggttgagatcaaaggcagcaccagcggctccggcaagcctggctctggcgagggcagcacaaagggacagctgcagctgcaggagtcgggcccaggactggtgaagccttcggagaccctgtccctcacctgcactgtctctggtggctccatcagcagtagtagttactactggggctggatccgccagcccccagggaaggggctggagtggattgggagtatctcctatagtgggagcacctactacaacccgtccctcaagagtcgagtcaccatatccgtagacacgtccaagaaccagttctccctgaagctgagttctgtgaccgccgcagacacggcggtgtactactgcgccagagatcgtggagacaccatactagacgtatggggtcagggtacaatggtcaccgtcagctca

SEQ ID NO: 45 - protein, 482 aa, Artificial Sequence
  CAR0009
DIVLTQSPPSLAMSLGKRATISCRASESVTILGSHLIHWYQQKPGQPPTLLIQLASNVQTGVPARFSGSGSRTDFTLTIDPVEEDDVAVYYCLQSRTIPRTFGGGTKLEIKGSTSGSGKPGSGEGSTKGQIQLVQSGPELKKPGETVKISCKASGYTFTDYSINWVKRAPGKGLKWMGWINTETREPAYAYDFRGRFAFSLETSASTAYLQINNLKYEDTATYFCALDYSYAMDYWGQGTSVTVSSFVPVFLPAKPTTTPAPRPPTPAPTIASQPLSLRPEACRPAAGGAVHTRGLDFACDIYIWAPLAGTCGVLLLSLVITLYCNHRNRSKRSRLLHSDYMNMTPRRPGPTRKHYQPYAPPRDFAAYRSRVKFSRSADAPAYQQGQNQLYNELNLGRREEYDVLDKRRGRDPEMGGKPRRKNPQEGLYNELQKDKMAEAYSEIGMKGERRRGKGHDGLYQGLSTATKDTYDALHMQALPPR

SEQ ID NO: 46 - DNA, 1446 bp, Artificial Sequence
  CAR0009 (nucleotide)
gacatcgtgctgacccagagcccccccagcctggccatgtctctgggcaagagagccaccatcagctgccgggccagcgagagcgtgaccatcctgggcagccacctgatccactggtatcagcagaagcccggccagccccccaccctgctgatccagctcgccagcaatgtgcagaccggcgtgcccgccagattcagcggcagcggcagcagaaccgacttcaccctgaccatcgaccccgtggaagaggacgacgtggccgtgtactactgcctgcagagccggaccatcccccggacctttggcggaggcaccaaactggaaatcaagggcagcaccagcggctccggcaagcctggctctggcgagggcagcacaaagggacagattcagctggtgcagagcggccctgagctgaagaaacccggcgagacagtgaagatcagctgcaaggcctccggctacaccttcaccgactacagcatcaactgggtgaaaagagcccctggcaagggcctgaagtggatgggctggatcaacaccgagacaagagagcccgcctacgcctacgacttccggggcagattcgccttcagcctggaaaccagcgccagcaccgcctacctgcagatcaacaacctgaagtacgaggacaccgccacctacttttgcgccctggactacagctacgccatggactactggggccagggcaccagcgtgaccgtgtccagcttcgtgcccgtgttcctgcccgccaaacctaccaccacccctgcccctagacctcccaccccagccccaacaatcgccagccagcctctgtctctgcggcccgaagcctgtagacctgctgccggcggagccgtgcacaccagaggcctggacttcgcctgcgacatctacatctgggcccctctggccggcacctgtggcgtgctgctgctgagcctggtgatcaccctgtactgcaaccaccggaacagaagcaagcggagccggctgctgcacagcgactacatgaacatgaccccaagacggcctggccccacccggaagcactaccagccttacgcccctcccagagacttcgccgcctaccggtccagagtgaagttcagcagatccgccgacgcccctgcctaccagcagggacagaaccagctgtacaacgagctgaacctgggcagacgggaagagtacgacgtgctggacaagcggagaggccgggaccccgagatgggcggaaagcccagacggaagaacccccaggaaggcctgtataacgaactgcagaaagacaagatggccgaggcctacagcgagatcggcatgaagggcgagcggaggcgcggcaagggccacgatggcctgtaccagggcctgagcaccgccaccaaggacacctacgacgccctgcacatgcaggccctgccccccaga

SEQ ID NO: 47 - protein, 491 aa, Artificial Sequence
  CAR0041
YPYDVPDYADIVLTQSPPSLAMSLGKRATISCRASESVTILGSHLIHWYQQKPGQPPTLLIQLASNVQTGVPARFSGSGSRTDFTLTIDPVEEDDVAVYYCLQSRTIPRTFGGGTKLEIKGSTSGSGKPGSGEGSTKGQIQLVQSGPELKKPGETVKISCKASGYTFTDYSINWVKRAPGKGLKWMGWINTETREPAYAYDFRGRFAFSLETSASTAYLQINNLKYEDTATYFCALDYSYAMDYWGQGTSVTVSSFVPVFLPAKPTTTPAPRPPTPAPTIASQPLSLRPEACRPAAGGAVHTRGLDFACDIYIWAPLAGTCGVLLLSLVITLYCNHRNRSKRSRLLHSDYMNMTPRRPGPTRKHYQPYAPPRDFAAYRSRVKFSRSADAPAYQQGQNQLYNELNLGRREEYDVLDKRRGRDPEMGGKPRRKNPQEGLYNELQKDKMAEAYSEIGMKGERRRGKGHDGLYQGLSTATKDTYDALHMQALPPR

SEQ ID NO: 48 - DNA, 1473 bp, Artificial Sequence
  CAR0041 (nucleotide)
tacccatacgatgttccagattacgctgacatcgtgctgacccagagcccccccagcctggccatgtctctgggcaagagagccaccatcagctgccgggccagcgagagcgtgaccatcctgggcagccacctgatccactggtatcagcagaagcccggccagccccccaccctgctgatccagctcgccagcaatgtgcagaccggcgtgcccgccagattcagcggcagcggcagcagaaccgacttcaccctgaccatcgaccccgtggaagaggacgacgtggccgtgtactactgcctgcagagccggaccatcccccggacctttggcggaggcaccaaactggaaatcaagggcagcaccagcggctccggcaagcctggctctggcgagggcagcacaaagggacagattcagctggtgcagagcggccctgagctgaagaaacccggcgagacagtgaagatcagctgcaaggcctccggctacaccttcaccgactacagcatcaactgggtgaaaagagcccctggcaagggcctgaagtggatgggctggatcaacaccgagacaagagagcccgcctacgcctacgacttccggggcagattcgccttcagcctggaaaccagcgccagcaccgcctacctgcagatcaacaacctgaagtacgaggacaccgccacctacttttgcgccctggactacagctacgccatggactactggggccagggcaccagcgtgaccgtgtccagcttcgtgcccgtgttcctgcccgccaaacctaccaccacccctgcccctagacctcccaccccagccccaacaatcgccagccagcctctgtctctgcggcccgaagcctgtagacctgctgccggcggagccgtgcacaccagaggcctggacttcgcctgcgacatctacatctgggcccctctggccggcacctgtggcgtgctgctgctgagcctggtgatcaccctgtactgcaaccaccggaacagaagcaagcggagccggctgctgcacagcgactacatgaacatgaccccaagacggcctggccccacccggaagcactaccagccttacgcccctcccagagacttcgccgcctaccggtccagagtgaagttcagcagatccgccgacgcccctgcctaccagcagggacagaaccagctgtacaacgagctgaacctgggcagacgggaagagtacgacgtgctggacaagcggagaggccgggaccccgagatgggcggaaagcccagacggaagaacccccaggaaggcctgtataacgaactgcagaaagacaagatggccgaggcctacagcgagatcggcatgaagggcgagcggaggcgcggcaagggccacgatggcctgtaccagggcctgagcaccgccaccaaggacacctacgacgccctgcacatgcaggccctgccccccaga

SEQ ID NO: 49 - protein, 488 aa, Artificial Sequence
  CAR0037
YPYDVPDYADIQMTQSPSSLSASVGDRVTITCRASQSISSYLNWYQQKPGKAPKLLIYAASSLQSGVPSRFSGSGSGTDFTLTISSLQPEDFATYYCQQKYDLLTFGGGTKVEIKGSTSGSGKPGSGEGSTKGQLQLQESGPGLVKPSETLSLTCTVSGGSISSSSYYWGWIRQPPGKGLEWIGSISYSGSTYYNPSLKSRVTISVDTSKNQFSLKLSSVTAADTAVYYCARDRGDTILDVWGQGTMVTVSSFVPVFLPAKPTTTPAPRPPTPAPTIASQPLSLRPEACRPAAGGAVHTRGLDFACDIYIWAPLAGTCGVLLLSLVITLYCNHRNRSKRSRLLHSDYMNMTPRRPGPTRKHYQPYAPPRDFAAYRSRVKFSRSADAPAYQQGQNQLYNELNLGRREEYDVLDKRRGRDPEMGGKPRRKNPQEGLYNELQKDKMAEAYSEIGMKGERRRGKGHDGLYQGLSTATKDTYDALHMQALPPR

SEQ ID NO: 50 - DNA, 1464 bp, Artificial Sequence
  CAR0037 (nucleotide)
tacccatacgatgttccagattacgctgacatccagatgacccagtctccatcctccctgtctgcatctgtaggagacagagtcaccatcacttgccgggcaagtcagagcattagcagctatttaaattggtatcagcagaaaccagggaaagcccctaagctcctgatctatgctgcatccagtttgcaaagtggggtcccatcaaggttcagtggcagtggatctgggacagatttcactctcaccatcagcagtctgcaacctgaagattttgcaacttactactgtcagcaaaaatacgacctcctcacttttggcggagggaccaaggttgagatcaaaggcagcaccagcggctccggcaagcctggctctggcgagggcagcacaaagggacagctgcagctgcaggagtcgggcccaggactggtgaagccttcggagaccctgtccctcacctgcactgtctctggtggctccatcagcagtagtagttactactggggctggatccgccagcccccagggaaggggctggagtggattgggagtatctcctatagtgggagcacctactacaacccgtccctcaagagtcgagtcaccatatccgtagacacgtccaagaaccagttctccctgaagctgagttctgtgaccgccgcagacacggcggtgtactactgcgccagagatcgtggagacaccatactagacgtatggggtcagggtacaatggtcaccgtcagctcattcgtgcccgtgttcctgcccgccaaacctaccaccacccctgcccctagacctcccaccccagccccaacaatcgccagccagcctctgtctctgcggcccgaagcctgtagacctgctgccggcggagccgtgcacaccagaggcctggacttcgcctgcgacatctacatctgggcccctctggccggcacctgtggcgtgctgctgctgagcctggtgatcaccctgtactgcaaccaccggaacagaagcaagcggagccggctgctgcacagcgactacatgaacatgaccccaagacggcctggccccacccggaagcactaccagccttacgcccctcccagagacttcgccgcctaccggtccagagtgaagttcagcagatccgccgacgcccctgcctaccagcagggacagaaccagctgtacaacgagctgaacctgggcagacgggaagagtacgacgtgctggacaagcggagaggccgggaccccgagatgggcggaaagcccagacggaagaacccccaggaaggcctgtataacgaactgcagaaagacaagatggccgaggcctacagcgagatcggcatgaagggcgagcggaggcgcggcaagggccacgatggcctgtaccagggcctgagcaccgccaccaaggacacctacgacgccctgcacatgcaggccctgccccccaga

SEQ ID NO: 51 - protein, 480 aa, Artificial Sequence
  CAR0085
DIQMTQSPSSLSASVGDRVTITCRASQSISSYLNWYQQKPGKAPKLLIYAASSLQSGVPSRFSGSGSGTDFTLTISSLQPEDFATYYCQQKYDLLTFGGGTKVEIKGSTSGSGKPGSGEGSTKGQLQLQESGPGLVKPSETLSLTCTVSGGSISSSSYYWGWIRQPPGKGLEWIGSISYSGSTYYNPSLKSRVTISVDTSKNQFSLKLSSVTAADTAVYYCARDRGDTILDVWGQGTMVTVSSFVPVFLPAKPTTTPAPRPPTPAPTIASQPLSLRPEACRPAAGGAVHTRGLDFACDIYIWAPLAGTCGVLLLSLVITLYCNHRNKRGRKKLLYIFKQPFMRPVQTTQEEDGCSCRFPEEEEGGCELRVKFSRSADAPAYQQGQNQLYNELNLGRREEYDVLDKRRGRDPEMGGKPRRKNPQEGLYNELQKDKMAEAYSEIGMKGERRRGKGHDGLYQGLSTATKDTYDALHMQALPPR

SEQ ID NO: 52 - DNA, 1440 bp, Artificial Sequence
  CAR0085 (nucleotide)
gacatccagatgacccagtctccatcctccctgtctgcatctgtaggagacagagtcaccatcacttgccgggcaagtcagagcattagcagctatttaaattggtatcagcagaaaccagggaaagcccctaagctcctgatctatgctgcatccagtttgcaaagtggggtcccatcaaggttcagtggcagtggatctgggacagatttcactctcaccatcagcagtctgcaacctgaagattttgcaacttactactgtcagcaaaaatacgacctcctcacttttggcggagggaccaaggttgagatcaaaggcagcaccagcggctccggcaagcctggctctggcgagggcagcacaaagggacagctgcagctgcaggagtcgggcccaggactggtgaagccttcggagaccctgtccctcacctgcactgtctctggtggctccatcagcagtagtagttactactggggctggatccgccagcccccagggaaggggctggagtggattgggagtatctcctatagtgggagcacctactacaacccgtccctcaagagtcgagtcaccatatccgtagacacgtccaagaaccagttctccctgaagctgagttctgtgaccgccgcagacacggcggtgtactactgcgccagagatcgtggagacaccatactagacgtatggggtcagggtacaatggtcaccgtcagctcattcgtgcccgtgttcctgcccgccaaacctaccaccacccctgcccctagacctcccaccccagccccaacaatcgccagccagcctctgtctctgcggcccgaagcctgtagacctgctgccggcggagccgtgcacaccagaggcctggacttcgcctgcgacatctacatctgggcccctctggccggcacctgtggcgtgctgctgctgagcctggtgatcaccctgtactgcaaccaccggaacaaacggggcagaaagaaactcctgtatatattcaaacaaccatttatgagaccagtacaaactactcaagaggaagatggctgtagctgccgatttccagaagaagaagaaggaggatgtgaactgagagtgaagttcagcagatccgccgacgcccctgcctaccagcagggacagaaccagctgtacaacgagctgaacctgggcagacgggaagagtacgacgtgctggacaagcggagaggccgggaccccgagatgggcggaaagcccagacggaagaacccccaggaaggcctgtataacgaactgcagaaagacaagatggccgaggcctacagcgagatcggcatgaagggcgagcggaggcgcggcaagggccacgatggcctgtaccagggcctgagcaccgccaccaaggacacctacgacgccctgcacatgcaggccctgccccccaga